European Patent Application EP 4 467 156 A1, published November 27, 2024. Title: A pharmaceutical composition for inhibiting fibrosis of organs. Applicant: Nagasaki University. The sequence listing filed with the application follows.

SEQUENCE LISTING (16 sequences)

SEQ ID NO: 1 - DNA, 19 bp, synthetic construct
  misc_feature 1..19: note = Primer
  source 1..19: mol_type = other DNA
cagaaaagggaccccagaa

SEQ ID NO: 2 - DNA, 23 bp, synthetic construct
  misc_feature 1..23: note = Primer
  source 1..23: mol_type = other DNA
gcagctgctctcgtagccatttc

SEQ ID NO: 3 - DNA, 23 bp, synthetic construct
  misc_feature 1..23: note = Primer
  source 1..23: mol_type = other DNA
aacatgctgctggataaatctgg

SEQ ID NO: 4 - DNA, 26 bp, synthetic construct
  misc_feature 1..26: note = Primer
  source 1..26: mol_type = other DNA
aggaaggcatggtacgatgtgataca

SEQ ID NO: 5 - DNA, 22 bp, synthetic construct
  misc_feature 1..22: note = Primer
  source 1..22: mol_type = other DNA
tcagaggtctacagatgaaggc

SEQ ID NO: 6 - DNA, 20 bp, synthetic construct
  misc_feature 1..20: note = Primer
  source 1..20: mol_type = other DNA
ccaggggctattggcaaagg

SEQ ID NO: 7 - DNA, 20 bp, synthetic construct
  misc_feature 1..20: note = Primer
  source 1..20: mol_type = other DNA
gtgacgaagcacagagcaaa

SEQ ID NO: 8 - DNA, 20 bp, synthetic construct
  misc_feature 1..20: note = Primer
  source 1..20: mol_type = other DNA
cttttccatgtcgtcccagt

SEQ ID NO: 9 - DNA, 23 bp, synthetic construct
  misc_feature 1..23: note = Primer
  source 1..23: mol_type = other DNA
cccaccaatcacctgcgtacaga

SEQ ID NO: 10 - DNA, 24 bp, synthetic construct
  misc_feature 1..24: note = Primer
  source 1..24: mol_type = other DNA
ttcttggtcggtgggtgactctga

SEQ ID NO: 11 - DNA, 22 bp, synthetic construct
  misc_feature 1..22: note = Primer
  source 1..22: mol_type = other DNA
tcttgatggtcgtctccaggta

SEQ ID NO: 12 - DNA, 22 bp, synthetic construct
  misc_feature 1..22: note = Primer
  source 1..22: mol_type = other DNA
gaggcggaagttctgttaggat

SEQ ID NO: 13 - DNA, 22 bp, synthetic construct
  misc_feature 1..22: note = Primer
  source 1..22: mol_type = other DNA
gactcatgaccacagtccatgc

SEQ ID NO: 14 - DNA, 21 bp, synthetic construct
  misc_feature 1..21: note = Primer
  source 1..21: mol_type = other DNA
agaggcagggatgatgttctg

SEQ ID NO: 15 - DNA, 22 bp, synthetic construct
  misc_feature 1..22: note = Primer
  source 1..22: mol_type = other DNA
tcaacaaaaatgagcacgcttt

SEQ ID NO: 16 - DNA, 21 bp, synthetic construct
  misc_feature 1..21: note = Primer
  source 1..21: mol_type = other DNA
aaacatggtgcaggcttcttg